European Patent Specification EP 3 655 554 B1, published October 30, 2024. Title: COMPOSITIONS AND METHODS FOR DETECTION OF BABESIA. Applicant: Roche Diagnostics GmbH F. Hoffmann-La Roche AG Roche Molecular Systems, Inc. The sequence listing filed with the application follows.

SEQUENCE LISTING (8 sequences)

SEQ ID NO: 1 - DNA, 23 bp, Artificial Sequence
  Forward Primer
  modified_base (23)..(23): t-Butyl Benzyl-dA
acctgctaaattaggatctggga

SEQ ID NO: 2 - DNA, 33 bp, Artificial Sequence
  Probe
  misc_feature (0)..(1): HEX-Thr
  misc_feature (10)..(11): BHQ-2
  misc_feature (33)..(34): Phosphate
ctgttccagtatcgcttcttagagggactttgc

SEQ ID NO: 3 - DNA, 24 bp, Artificial Sequence
  Reverse Primer
  modified_base (24)..(24): t-Butyl Benzyl-dC
tgttattgccttacacttccttgc

SEQ ID NO: 4 - DNA, 16 bp, Artificial Sequence
  Forward Primer
  modified_base (16)..(16): t-Butyl Benzyl-dA
gatgtcctgggctgca

SEQ ID NO: 5 - DNA, 28 bp, Artificial Sequence
  Probe
  misc_feature (0)..(1): HEX-Thr
  misc_feature (8)..(9): BHQ-2
  misc_feature (29)..(30): Phosphate
aactcgatgaatgcatcagtgtagcgcg

SEQ ID NO: 6 - DNA, 22 bp, Artificial Sequence
  Reverse Primer
  modified_base (22)..(22): t-Butyl Benzyl-dA
ccccgtcacgatgcatactaaa

SEQ ID NO: 7 - DNA, 22 bp, Artificial Sequence
  Reverse Primer
  modified_base (22)..(22): t-Butyl Benzyl-dA
ccccatcacgatgcatactaaa

SEQ ID NO: 8 - DNA, 419 bp, Artificial Sequence
  Positive Control
gattagatctaattccaccaggtccagacatagagaggattgacagattgatagctctttcttgattctatgggtggtggtgcatggccgttcttagttggtggagtgatttgtctggttaattccgttaacgaacgagaccttaacctgctaaattaggatctgggacaagctttgctgttccagtatcgcttcttagagggactttgcgttcataaaacgcaaggaagtgtaaggcaataacaggtctgtgatgcccttagatgtcctgggctgcacgcgcgctacactgatgcattcaacgagtttttccttggccgtcgggtccgggtaatcttacagtatgcatcgtgatggggatagattattgcaattattaatcttgaaacatgaggattacccatgtctcgaggtgtaat